European Patent Application EP 4 268 847 A1, published November 1, 2023. Title: A pharmaceutical composition for treating amyotrophic lateral sclerosis. Applicant: EISAI R&D MANAGEMENT CO., LTD. The sequence listing filed with the application follows.

SEQUENCE LISTING (66 sequences)

SEQ ID NO: 1 - protein, 986 aa, Mus musculus
MAGIFYFILFSFLFGICDAVTGSRVYPANEVTLLDSRSVQGELGWIASPLEGGWEEVSIMDEKNTPIRTYQVCNVMEASQNNWLRTDWITREGAQRVYIEIKFTLRDCNSLPGVMGTCKETFNLYYYESDNDKERFIRESQFGKIDTIAADESFTQVDIGDRIMKLNTEIRDVGPLSKKGFYLAFQDVGACIALVSVRVFYKKCPLTVRNLAQFPDTITGADTSSLVEVRGSCVNNSEEKDVPKMYCGADGEWLVPIGNCLCNAGHEEQNGECQACKIGYYKALSTDASCAKCPPHSYSVWEGATSCTCDRGFFRADNDAASMPCTRPPSAPLNLISNVNETSVNLEWSSPQNTGGRQDISYNVVCKKCGAGDPSKCRPCGSGVHYTPQQNGLKTTRVSITDLLAHTNYTFEIWAVNGVSKYNPSPDQSVSVTVTTNQAAPSSIALVQAKEVTRYSVALAWLEPDRPNGVILEYEVKYYEKDQNERSYRIVRTAARNTDIKGLNPLTSYVFHVRARTAAGYGDFSEPLEVTTNTVPSRIIGDGANSTVLLVSVSGSVVLVVILIAAFVISRRRSKYSKAKQEADEEKHLNQGVRTYVDPFTYEDPNQAVREFAKEIDASCIKIEKVIGVGEFGEVCSGRLKVPGKREICVAIKTLKAGYTDKQRRDFLSEASIMGQFDHPNIIHLEGVVTKCKPVMIITEYMENGSLDAFLRKNDGRFTVIQLVGMLRGIGSGMKYLSDMSYVHRDLAARNILVNSNLVCKVSDFGMSRVLEDDPEAAYTTRGGKIPIRWTAPEAIAYRKFTSASDVWSYGIVMWEVMSYGERPYWDMSNQDVIKAIEEGYRLPPPMDCPIALHQLMLDCWQKERSDRPKFGQIVNMLDKLIRNPNSLKRTGSESSRPNTALLDPSSPEFSAVVSVGDWLQAIKMDRYKDNFTAAGYTTLEAVVHMSQDDLARIGITAITHQNKILSSVQAMRTQMQQMHGRMVPV

SEQ ID NO: 2 - protein, 528 aa, Mus musculus
VTGSRVYPANEVTLLDSRSVQGELGWIASPLEGGWEEVSIMDEKNTPIRTYQVCNVMEASQNNWLRTDWITREGAQRVYIEIKFTLRDCNSLPGVMGTCKETFNLYYYESDNDKERFIRESQFGKIDTIAADESFTQVDIGDRIMKLNTEIRDVGPLSKKGFYLAFQDVGACIALVSVRVFYKKCPLTVRNLAQFPDTITGADTSSLVEVRGSCVNNSEEKDVPKMYCGADGEWLVPIGNCLCNAGHEEQNGECQACKIGYYKALSTDASCAKCPPHSYSVWEGATSCTCDRGFFRADNDAASMPCTRPPSAPLNLISNVNETSVNLEWSSPQNTGGRQDISYNVVCKKCGAGDPSKCRPCGSGVHYTPQQNGLKTTRVSITDLLAHTNYTFEIWAVNGVSKYNPSPDQSVSVTVTTNQAAPSSIALVQAKEVTRYSVALAWLEPDRPNGVILEYEVKYYEKDQNERSYRIVRTAARNTDIKGLNPLTSYVFHVRARTAAGYGDFSEPLEVTTNTVPSRIIGDGANST

SEQ ID NO: 3 - protein, 1030 aa, Artificial Sequence
  Synthetic polypeptide
VTGSRVYPANEVTLLDSRSVQGELGWIASPLEGGWEEVSIMDEKNTPIRTYQVCNVMEASQNNWLRTDWITREGAQRVYIEIKFTLRDCNSLPGVMGTCKETFNLYYYESDNDKERFIRESQFGKIDTIAADESFTQVDIGDRIMKLNTEIRDVGPLSKKGFYLAFQDVGACIALVSVRVFYKKCPLTVRNLAQFPDTITGADTSSLVEVRGSCVNNSEEKDVPKMYCGADGEWLVPIGNCLCNAGHEEQNGECQACKIGYYKALSTDASCAKCPPHSYSVWEGATSCTCDRGFFRADNDAASMPCTRPPSAPLNLISNVNETSVNLEWSSPQNTGGRQDISYNVVCKKCGAGDPSKCRPCGSGVHYTPQQNGLKTTRVSITDLLAHTNYTFEIWAVNGVSKYNPSPDQSVSVTVTTNQAAPSSIALVQAKEVTRYSVALAWLEPDRPNGVILEYEVKYYEKDQNERSYRIVRTAARNTDIKGLNPLTSYVFHVRARTAAGYGDFSEPLEVTTNTVPSRIIGDGANSTAAAIIPVEEENPDFWNREAAEALGAAKKLQPAQTAAKNLIIFLGDGMGVSTVTAARILKGQKKDKLGPEIPLAMDRFPYVALSKTYNVDKHVPDSGATATAYLCGVKGNFQTIGLSAAARFNQCNTTRGNEVISVMNRAKKAGKSVGVVTTTRVQHASPAGTYAHTVNRNWYSDADVPASARQEGCQDIATQLISNMDIDVILGGGRKYMFRMGTPDPEYPDDYSQGGTRLDGKNLVQEWLAKRQGARYVWNRTELMQASLDPSVTHLMGLFEPGDMKYEIHRDSTLDPSLMEMTEAALRLLSRNPRGFFLFVEGGRIDHGHHESRAYRALTETIMFDDAIERAGQLTSEEDTLSLVTADHSHVFSFGGYPLRGSSIFGLAPGKARDRKAYTVLLYGNGPGYVLKDGARPDVTESESGSPEYRQQSAVPLDEETHAGEDVAVFARGPQAHLVHGVQEQTFIAHVMAFAACLEPYTACDLAPPAGTTDAAHPGHHHHHHHHHH

SEQ ID NO: 4 - protein, 19 aa, Mus musculus
MAGIFYFILFSFLFGICDA

SEQ ID NO: 5 - protein, 986 aa, Homo sapiens
MAGIFYFALFSCLFGICDAVTGSRVYPANEVTLLDSRSVQGELGWIASPLEGGWEEVSIMDEKNTPIRTYQVCNVMEPSQNNWLRTDWITREGAQRVYIEIKFTLRDCNSLPGVMGTCKETFNLYYYESDNDKERFIRENQFVKIDTIAADESFTQVDIGDRIMKLNTEIRDVGPLSKKGFYLAFQDVGACIALVSVRVFYKKCPLTVRNLAQFPDTITGADTSSLVEVRGSCVNNSEEKDVPKMYCGADGEWLVPIGNCLCNAGHEERSGECQACKIGYYKALSTDATCAKCPPHSYSVWEGATSCTCDRGFFRADNDAASMPCTRPPSAPLNLISNVNETSVNLEWSSPQNTGGRQDISYNVVCKKCGAGDPSKCRPCGSGVHYTPQQNGLKTTKVSITDLLAHTNYTFEIWAVNGVSKYNPNPDQSVSVTVTTNQAAPSSIALVQAKEVTRYSVALAWLEPDRPNGVILEYEVKYYEKDQNERSYRIVRTAARNTDIKGLNPLTSYVFHVRARTAAGYGDFSEPLEVTTNTVPSRIIGDGANSTVLLVSVSGSVVLVVILIAAFVISRRRSKYSKAKQEADEEKHLNQGVRTYVDPFTYEDPNQAVREFAKEIDASCIKIEKVIGVGEFGEVCSGRLKVPGKREICVAIKTLKAGYTDKQRRDFLSEASIMGQFDHPNIIHLEGVVTKCKPVMIITEYMENGSLDAFLRKNDGRFTVIQLVGMLRGIGSGMKYLSDMSYVHRDLAARNILVNSNLVCKVSDFGMSRVLEDDPEAAYTTRGGKIPIRWTAPEAIAYRKFTSASDVWSYGIVMWEVMSYGERPYWDMSNQDVIKAIEEGYRLPPPMDCPIALHQLMLDCWQKERSDRPKFGQIVNMLDKLIRNPNSLKRTGTESSRPNTALLDPSSPEFSAVVSVGDWLQAIKMDRYKDNFTAAGYTTLEAVVHVNQEDLARIGITAITHQNKILSSVQAMRTQMQQMHGRMVPV

SEQ ID NO: 6 - protein, 528 aa, Homo sapiens
VTGSRVYPANEVTLLDSRSVQGELGWIASPLEGGWEEVSIMDEKNTPIRTYQVCNVMEPSQNNWLRTDWITREGAQRVYIEIKFTLRDCNSLPGVMGTCKETFNLYYYESDNDKERFIRENQFVKIDTIAADESFTQVDIGDRIMKLNTEIRDVGPLSKKGFYLAFQDVGACIALVSVRVFYKKCPLTVRNLAQFPDTITGADTSSLVEVRGSCVNNSEEKDVPKMYCGADGEWLVPIGNCLCNAGHEERSGECQACKIGYYKALSTDATCAKCPPHSYSVWEGATSCTCDRGFFRADNDAASMPCTRPPSAPLNLISNVNETSVNLEWSSPQNTGGRQDISYNVVCKKCGAGDPSKCRPCGSGVHYTPQQNGLKTTKVSITDLLAHTNYTFEIWAVNGVSKYNPNPDQSVSVTVTTNQAAPSSIALVQAKEVTRYSVALAWLEPDRPNGVILEYEVKYYEKDQNERSYRIVRTAARNTDIKGLNPLTSYVFHVRARTAAGYGDFSEPLEVTTNTVPSRIIGDGANST

SEQ ID NO: 7 - DNA, 12 bp, Artificial Sequence
  ad29S
acatcactccgt

SEQ ID NO: 8 - DNA, 50 bp, Artificial Sequence
  ad29AS
acggagtgatgtccgtcgacgtatctctgcgttgatacttcagcgtagct

SEQ ID NO: 9 - DNA, 26 bp, Artificial Sequence
  Synthetic primer
agctacgctgaagtatcaacgcagag

SEQ ID NO: 10 - DNA, 20 bp, Artificial Sequence
  Synthetic primer
gccagtggatagactgatgg

SEQ ID NO: 11 - DNA, 21 bp, Artificial Sequence
  Synthetic primer
gatggatacagttggtgcagc

SEQ ID NO: 12 - protein, 19 aa, Artificial Sequence
  Synthetic polypeptide
MAVLVLLLCLVTFPSCVLS

SEQ ID NO: 13 - protein, 125 aa, Artificial Sequence
  Synthetic polypeptide
QVQLKQSGPSLVQPSQSLSITCTVSGFSLTRYGVHWVRQSPGKGLEWLGVIWRGGSTDYNAAFMSRLSITKDNSKSQVFFKMNSLQADDTAIYYCAKESLFGVYYDYGYYSMDYWGQGTSVTVSS

SEQ ID NO: 14 - protein, 22 aa, Artificial Sequence
  Synthetic polypeptide
MDMRVPAHVFGFLLLWFPGTRC

SEQ ID NO: 15 - protein, 107 aa, Artificial Sequence
  Synthetic polypeptide
DIQMTQSPSSLSASLGERVSLTCRASQEISGYLSWLQQKPDGTIKRLIYAASTLDSGVPKRFSGSRSGSDYSLTISSLESEDFADYYCLQYASYPLTFGAGTKLELK

SEQ ID NO: 16 - DNA, 57 bp, Artificial Sequence
  Synthetic polynucleotide
atggctgtcctggtgctgctcctctgcctggtgacattcccaagctgtgtcctgtcc

SEQ ID NO: 17 - DNA, 375 bp, Artificial Sequence
  Synthetic polynucleotide
caggtgcagctgaagcagtcaggacctagcctagtgcagccctcacagagcctgtccataacctgcacagtctctggtttctcattaactaggtatggtgtacactgggttcgccagtctccaggaaagggtctggagtggctgggagtgatttggagaggtggaagcacagactacaatgcagctttcatgtccagactgagcatcaccaaggacaactccaagagccaagttttctttaaaatgaacagtctgcaagctgatgacactgccatatactactgtgccaaagaaagcctatttggggtctactatgattacgggtactattctatggactactggggtcaaggaacctcagtcaccgtctcctca

SEQ ID NO: 18 - DNA, 66 bp, Artificial Sequence
  Synthetic polynucleotide
atggacatgagggttcctgctcacgtttttggcttcttgttgctctggtttccaggtaccagatgt

SEQ ID NO: 19 - DNA, 321 bp, Artificial Sequence
  Synthetic polynucleotide
gacatccaaatgacccagtctccatcctccttatctgcctctctgggagaaagagtcagtctcacttgtcgggcaagtcaggaaattagtggttacttaagctggcttcagcagaaaccagatggaactattaaacgcctgatctacgccgcatccactttagattctggtgtcccaaaaaggttcagtggcagtaggtctgggtcagattattctctcaccatcagcagccttgagtctgaagattttgcagactattactgtctacaatatgctagttatccgctcacgttcggtgctgggaccaagctggagctgaaa

SEQ ID NO: 20 - DNA, 40 bp, Artificial Sequence
  Synthetic primer
gcgaagcttgccgccaccatggctgtcctggtgctgctcc

SEQ ID NO: 21 - DNA, 43 bp, Artificial Sequence
  Synthetic primer
gcgaagcttgccgccaccatggacatgagggttcctgctcacg

SEQ ID NO: 22 - DNA, 36 bp, Artificial Sequence
  Synthetic primer
gcggaattcatcatttaccaggagagtgggagaggc

SEQ ID NO: 23 - DNA, 40 bp, Artificial Sequence
  Synthetic primer
cgcgaattcactaacactcattcctgttgaagctcttgac

SEQ ID NO: 24 - protein, 324 aa, Artificial Sequence
  Synthetic polypeptide
AKTTPPSVYPLAPGSAAQTNSMVTLGCLVKGYFPEPVTVTWNSGSLSSGVHTFPAVLQSDLYTLSSSVTVPSSTWPSETVTCNVAHPASSTKVDKKIVPRDCGCKPCICTVPEVSSVFIFPPKPKDVLTITLTPKVTCVVVDISKDDPEVQFSWFVDDVEVHTAQTQPREEQFNSTFRSVSELPIMHQDWLNGKEFKCRVNSAAFPAPIEKTISKTKGRPKAPQVYTIPPPKEQMAKDKVSLTCMITDFFPEDITVEWQWNGQPAENYKNTQPIMDTDGSYFVYSKLNVQKSNWEAGNTFTCSVLHEGLHNHHTEKSLSHSPGK

SEQ ID NO: 25 - protein, 107 aa, Artificial Sequence
  Synthetic polypeptide
RADAAPTVSIFPPSSEQLTSGGASVVCFLNNFYPKDINVKWKIDGSERQNGVLNSWTDQDSKDSTYSMSSTLTLTKDEYERHNSYTCEATHKTSTSPIVKSFNRNEC

SEQ ID NO: 26 - protein, 5 aa, Artificial Sequence
  Synthetic peptide
RYGVH

SEQ ID NO: 27 - protein, 16 aa, Artificial Sequence
  Synthetic peptide
VIWRGGSTDYNAAFMS

SEQ ID NO: 28 - protein, 17 aa, Artificial Sequence
  Synthetic peptide
ESLFGVYYDYGYYSMDY

SEQ ID NO: 29 - protein, 11 aa, Artificial Sequence
  Synthetic peptide
RASQEISGYLS

SEQ ID NO: 30 - protein, 7 aa, Artificial Sequence
  Synthetic peptide
AASTLDS

SEQ ID NO: 31 - protein, 9 aa, Artificial Sequence
  Synthetic peptide
LQYASYPLT

SEQ ID NO: 32 - protein, 986 aa, Macaca mulatta
MAGIFYFALFSCLFGICDAVTGSRVYPANEVTLLDSRSVQGELGWIASPLEGGWEEVSIMDEKNTPIRTYQVCNVMEPSQNNWLRTDWITREGAQRVYIEIKFTLRDCNSLPGVMGTCKETFNLYYYESDNDKERFIRENQFVKIDTIAADESFTQVDIGDRIMKLNTEIRDVGPLSKKGFYLAFQDVGACIALVSVRVFYKKCPLTVRNLAQFPDTITGADTSSLVEVRGSCVNNSEEKDVPKMYCGADGEWLVPIGNCLCNAGHEERSGECQACKIGYYKALSTDATCAKCPPHSYSVWEGATSCTCDRGFFRADNDAASMPCTRPPSAPLNLISNVNETSVNLEWSSPQNTGGRQDISYNVVCKKCGAGDPSKCRPCGSGVHYTPQQNGLKTTKVSITDLLAHTNYTFEIWAVNGVSKYNPSPDQSVSVTVTTNQAAPSSIALVQAKEVTRYSVALAWLEPDRPNGVILEYEVKYYEKDQNERSYRIVRTAARNTDIKGLNPLTSYVFHVRARTAAGYGDFSEPLEVTTNTVPSRIIGDGANSTVLLVSVSGSVVLVVILIAAFVISRRRSKYSKAKQEADEEKHLNQGVRTYVDPFTYEDPNQAVREFAKEIDASCIKIEKVIGVGEFGEVCSGRLKVPGKREICVAIKTLKAGYTDKQRRDFLSEASIMGQFDHPNIIHLEGVVTKCKPVMIITEYMENGSLDAFLRKNDGRFTVIQLVGMLRGIGSGMKYLSDMSYVHRDLAARNILVNSNLVCKVSDFGMSRVLEDDPEAAYTTRGGKIPIRWTAPEAIAYRKFTSASDVWSYGIVMWEVMSYGERPYWDMSNQDVIKAIEEGYRLPPPMDCPIALHQLMLDCWQKERSDRPKFGQIVNMLDKLIRNPNSLKRTGTESSRPNTALLDPSSPEFSAVVSVGDWLQAIKMDRYKDNFTAAGYTTLEAVVHVNQEDLARIGITAITHQNKILSSVQAMRTQMQQMHGRMVPV

SEQ ID NO: 33 - protein, 528 aa, Macaca mulatta
VTGSRVYPANEVTLLDSRSVQGELGWIASPLEGGWEEVSIMDEKNTPIRTYQVCNVMEPSQNNWLRTDWITREGAQRVYIEIKFTLRDCNSLPGVMGTCKETFNLYYYESDNDKERFIRENQFVKIDTIAADESFTQVDIGDRIMKLNTEIRDVGPLSKKGFYLAFQDVGACIALVSVRVFYKKCPLTVRNLAQFPDTITGADTSSLVEVRGSCVNNSEEKDVPKMYCGADGEWLVPIGNCLCNAGHEERSGECQACKIGYYKALSTDATCAKCPPHSYSVWEGATSCTCDRGFFRADNDAASMPCTRPPSAPLNLISNVNETSVNLEWSSPQNTGGRQDISYNVVCKKCGAGDPSKCRPCGSGVHYTPQQNGLKTTKVSITDLLAHTNYTFEIWAVNGVSKYNPSPDQSVSVTVTTNQAAPSSIALVQAKEVTRYSVALAWLEPDRPNGVILEYEVKYYEKDQNERSYRIVRTAARNTDIKGLNPLTSYVFHVRARTAAGYGDFSEPLEVTTNTVPSRIIGDGANST

SEQ ID NO: 34 - protein, 19 aa, Homo sapiens
MAGIFYFALFSCLFGICDA

SEQ ID NO: 35 - protein, 15 aa, Homo sapiens
MSALLILALVGAAVA

SEQ ID NO: 36 - protein, 547 aa, Homo sapiens
MAGIFYFALFSCLFGICDAVTGSRVYPANEVTLLDSRSVQGELGWIASPLEGGWEEVSIMDEKNTPIRTYQVCNVMEPSQNNWLRTDWITREGAQRVYIEIKFTLRDCNSLPGVMGTCKETFNLYYYESDNDKERFIRENQFVKIDTIAADESFTQVDIGDRIMKLNTEIRDVGPLSKKGFYLAFQDVGACIALVSVRVFYKKCPLTVRNLAQFPDTITGADTSSLVEVRGSCVNNSEEKDVPKMYCGADGEWLVPIGNCLCNAGHEERSGECQACKIGYYKALSTDATCAKCPPHSYSVWEGATSCTCDRGFFRADNDAASMPCTRPPSAPLNLISNVNETSVNLEWSSPQNTGGRQDISYNVVCKKCGAGDPSKCRPCGSGVHYTPQQNGLKTTKVSITDLLAHTNYTFEIWAVNGVSKYNPNPDQSVSVTVTTNQAAPSSIALVQAKEVTRYSVALAWLEPDRPNGVILEYEVKYYEKDQNERSYRIVRTAARNTDIKGLNPLTSYVFHVRARTAAGYGDFSEPLEVTTNTVPSRIIGDGANST

SEQ ID NO: 37 - protein, 328 aa, Homo sapiens
MAGIFYFALFSCLFGICDAVTGSRVYPANEVTLLDSRSVQGELGWIASPLEGGWEEVSIMDEKNTPIRTYQVCNVMEPSQNNWLRTDWITREGAQRVYIEIKFTLRDCNSLPGVMGTCKETFNLYYYESDNDKERFIRENQFVKIDTIAADESFTQVDIGDRIMKLNTEIRDVGPLSKKGFYLAFQDVGACIALVSVRVFYKKCPLTVRNLAQFPDTITGADTSSLVEVRGSCVNNSEEKDVPKMYCGADGEWLVPIGNCLCNAGHEERSGECQACKIGYYKALSTDATCAKCPPHSYSVWEGATSCTCDRGFFRADNDAASMPCTRP

SEQ ID NO: 38 - protein, 236 aa, Homo sapiens
PLTVRNLAQFPDTITGADTSSLVEVRGSCVNNSEEKDVPKMYCGADGEWLVPIGNCLCNAGHEERSGECQACKIGYYKALSTDATCAKCPPHSYSVWEGATSCTCDRGFFRADNDAASMPCTRPPSAPLNLISNVNETSVNLEWSSPQNTGGRQDISYNVVCKKCGAGDPSKCRPCGSGVHYTPQQNGLKTTKVSITDLLAHTNYTFEIWAVNGVSKYNPNPDQSVSVTVTTNQAA

SEQ ID NO: 39 - protein, 112 aa, Homo sapiens
TNQAAPSSIALVQAKEVTRYSVALAWLEPDRPNGVILEYEVKYYEKDQNERSYRIVRTAARNTDIKGLNPLTSYVFHVRARTAAGYGDFSEPLEVTTNTVPSRIIGDGANST

SEQ ID NO: 40 - protein, 96 aa, Artificial Sequence
  Synthetic polypeptide
DIQMTQSPSSLSASVGDRVTITCRASQGIRNDLGWYQQKPGKAPKRLIYAASSLQSGVPSRFSGSGSGTEFTLTISSLQPEDFATYYCLQHNSYPP

SEQ ID NO: 41 - protein, 12 aa, Artificial Sequence
  Synthetic polypeptide
LTFGGGTKVEIK

SEQ ID NO: 42 - protein, 98 aa, Artificial Sequence
  Synthetic polypeptide
QVQLVESGGGVVQPGRSLRLSCAASGFTFSSYGMHWVRQAPGKGLEWVAVIWYDGSNKYYADSVKGRFTISRDNSKNTLYLQMNSLRAEDTAVYYCAK

SEQ ID NO: 43 - protein, 18 aa, Artificial Sequence
  Synthetic polypeptide
YYYYGMDVWGQGTTVTVS

SEQ ID NO: 44 - protein, 5 aa, Artificial Sequence
  Synthetic polypeptide
RFGVH

SEQ ID NO: 45 - protein, 125 aa, Artificial Sequence
  Synthetic polypeptide
QVQLVESGGGVVQPGRSLRLSCAVSGFSLTRFGVHWVRQAPGKGLEWVAVIWRGGSTDYNAAFMSRLTISKDNSKNTVYLQMNSLRAEDTAVYYCAKESLFGVYYDYGYYSMDYWGQGTTVTVSS

SEQ ID NO: 46 - protein, 107 aa, Artificial Sequence
  Synthetic polypeptide
DIQMTQSPSSLSASVGDRVTITCRASQEISGYLSWLQQKPGKAPKRLIYAASTLDSGVPSRFSGSRSGTEYTLTISSLQPEDFATYYCLQYASYPLTFGGGTKVEIK

SEQ ID NO: 47 - protein, 326 aa, Homo sapiens
ASTKGPSVFPLAPSSRSTSESTAALGCLVKDYFPEPVTVSWNSGALTSGVHTFPAVLQSSGLYSLSSVVTVPSSNFGTQTYTCNVDHKPSNTKVDKTVERKSCVECPPCPAPPAAAPSVFLFPPKPKDTLMISRTPEVTCVVVDVSHEDPEVQFNWYVDGVEVHNAKTKPREEQFNSTFRVVSVLTVVHQDWLNGKEYKCKVSNKGLPAPIEKTISKTKGQPREPQVYTLPPSREEMTKNQVSLTCLVKGFYPSDIAVEWESNGQPENNYKTTPPMLDSDGSFFLYSKLTVDKSRWQQGNVFSCSVMHEALHNHYTQKSLSLSPGK

SEQ ID NO: 48 - protein, 107 aa, Homo sapiens [sequence omitted]

SEQ ID NO: 49 - DNA, 15 bp, Artificial Sequence
  Synthetic polynucleotide
agatttggagtgcat

SEQ ID NO: 50 - DNA, 48 bp, Artificial Sequence
  Synthetic polynucleotide
gtgatctggaggggaggatccaccgactacaacgctgcttttatgagc

SEQ ID NO: 51 - DNA, 51 bp, Artificial Sequence
  Synthetic polynucleotide
gagagcctgttcggcgtgtactatgactacggctactattctatggattat

SEQ ID NO: 52 - DNA, 33 bp, Artificial Sequence
  Synthetic polynucleotide
cgcgcctcccaggagatctctggctacctgtcc

SEQ ID NO: 53 - DNA, 21 bp, Artificial Sequence
  Synthetic polynucleotide
gctgcctccaccctggactct

SEQ ID NO: 54 - DNA, 27 bp, Artificial Sequence
  Synthetic polynucleotide
ctgcagtacgcttcctatccactgacc

SEQ ID NO: 55 - DNA, 375 bp, Artificial Sequence
  Synthetic polynucleotide
caggtgcagctggtggagagcggaggaggagtggtgcagcctggcaggtccctgaggctgagctgtgccgtgtccggcttcagcctgacaagatttggagtgcattgggtgcgccaggctccaggcaagggactggagtgggtggccgtgatctggaggggaggatccaccgactacaacgctgcttttatgagccggctgacaatctctaaggataactccaagaataccgtgtatctgcagatgaactccctgagggctgaggacaccgccgtgtactattgcgccaaggagagcctgttcggcgtgtactatgactacggctactattctatggattattggggccagggcaccacagtgacagtgtcctcc

SEQ ID NO: 56 - DNA, 321 bp, Artificial Sequence
  Synthetic polynucleotide
gatatccagatgacacagtccccttccagcctgtctgcctccgtgggcgacagagtgaccatcacatgtcgcgcctcccaggagatctctggctacctgtcctggctgcagcagaagccaggcaaggctcccaagcgcctgatctatgctgcctccaccctggactctggagtgccttccaggttcagcggctctcggtccggcacagagtacaccctgacaatctcttccctgcagcctgaggatttcgccacctactattgcctgcagtacgcttcctatccactgacctttggcggcggcacaaaggtggagatcaag

SEQ ID NO: 57 - DNA, 978 bp, Artificial Sequence
  Synthetic polynucleotide
gcctccaccaagggaccatccgtgttcccactggccccatcttcccggagcacatctgagtccaccgccgctctgggctgtctggtgaaggattacttccctgagccagtgacagtgtcttggaactccggcgctctgacatccggcgtgcacacctttcctgccgtgctgcagagctctggcctgtacagcctgtccagcgtggtgaccgtgccctcttccaatttcggcacccagacatatacctgcaacgtggaccataagccttccaatacaaaggtggataagaccgtggagagaaagagctgcgtggagtgtccaccttgcccagctccaccagccgctgcccctagcgtgttcctgtttcctccaaagccaaaggacacactgatgatctctcgcacacccgaggtgacctgcgtggtggtggacgtgtcccacgaggatccagaggtgcagtttaactggtacgtggatggcgtggaggtgcataatgctaagaccaagcccagggaggagcagttcaactccacatttcgggtggtgagcgtgctgaccgtggtgcaccaggactggctgaacggcaaggagtataagtgtaaggtgagcaataagggcctgcccgcccctatcgagaagacaatctctaagaccaagggccagcctagagagccacaggtgtacaccctgcccccttctcgcgaggagatgacaaagaaccaggtgtccctgacctgcctggtgaagggcttctatcctagcgacatcgctgtggagtgggagtctaatggccagccagagaacaattacaagaccacaccacccatgctggacagcgatggctctttctttctgtattctaagctgacagtggataagtccaggtggcagcagggcaacgtgtttagctgctctgtgatgcatgaggccctgcacaatcattacacccagaagtccctgagcctgtctccaggcaag

SEQ ID NO: 58 - DNA, 321 bp, Artificial Sequence
  Synthetic polynucleotide
aggacagtggccgctccatccgtgttcatctttccccctagcgacgagcagctgaagagcggcaccgcctctgtggtgtgcctgctgaacaatttctaccccagggaggccaaggtgcagtggaaggtggataacgctctgcagagcggcaattctcaggagtccgtgaccgagcaggacagcaaggattctacatattccctgagctctaccctgacactgagcaaggccgattacgagaagcacaaggtgtatgcttgcgaggtgacccatcagggcctgtccagcccagtgacaaagtcttttaacaggggcgagtgt

SEQ ID NO: 59 - protein, 451 aa, Artificial Sequence
  Synthetic polypeptide
QVQLVESGGGVVQPGRSLRLSCAVSGFSLTRFGVHWVRQAPGKGLEWVAVIWRGGSTDYNAAFMSRLTISKDNSKNTVYLQMNSLRAEDTAVYYCAKESLFGVYYDYGYYSMDYWGQGTTVTVSSASTKGPSVFPLAPSSRSTSESTAALGCLVKDYFPEPVTVSWNSGALTSGVHTFPAVLQSSGLYSLSSVVTVPSSNFGTQTYTCNVDHKPSNTKVDKTVERKSCVECPPCPAPPAAAPSVFLFPPKPKDTLMISRTPEVTCVVVDVSHEDPEVQFNWYVDGVEVHNAKTKPREEQFNSTFRVVSVLTVVHQDWLNGKEYKCKVSNKGLPAPIEKTISKTKGQPREPQVYTLPPSREEMTKNQVSLTCLVKGFYPSDIAVEWESNGQPENNYKTTPPMLDSDGSFFLYSKLTVDKSRWQQGNVFSCSVMHEALHNHYTQKSLSLSPGK

SEQ ID NO: 60 - protein, 214 aa, Artificial Sequence
  Synthetic polypeptide
DIQMTQSPSSLSASVGDRVTITCRASQEISGYLSWLQQKPGKAPKRLIYAASTLDSGVPSRFSGSRSGTEYTLTISSLQPEDFATYYCLQYASYPLTFGGGTKVEIKRTVAAPSVFIFPPSDEQLKSGTASVVCLLNNFYPREAKVQWKVDNALQSGNSQESVTEQDSKDSTYSLSSTLTLSKADYEKHKVYACEVTHQGLSSPVTKSFNRGEC

SEQ ID NO: 61 - DNA, 1353 bp, Artificial Sequence
  Synthetic polynucleotide
caggtgcagctggtggagagcggaggaggagtggtgcagcctggcaggtccctgaggctgagctgtgccgtgtccggcttcagcctgacaagatttggagtgcattgggtgcgccaggctccaggcaagggactggagtgggtggccgtgatctggaggggaggatccaccgactacaacgctgcttttatgagccggctgacaatctctaaggataactccaagaataccgtgtatctgcagatgaactccctgagggctgaggacaccgccgtgtactattgcgccaaggagagcctgttcggcgtgtactatgactacggctactattctatggattattggggccagggcaccacagtgacagtgtcctccgcctccaccaagggaccatccgtgttcccactggccccatcttcccggagcacatctgagtccaccgccgctctgggctgtctggtgaaggattacttccctgagccagtgacagtgtcttggaactccggcgctctgacatccggcgtgcacacctttcctgccgtgctgcagagctctggcctgtacagcctgtccagcgtggtgaccgtgccctcttccaatttcggcacccagacatatacctgcaacgtggaccataagccttccaatacaaaggtggataagaccgtggagagaaagagctgcgtggagtgtccaccttgcccagctccaccagccgctgcccctagcgtgttcctgtttcctccaaagccaaaggacacactgatgatctctcgcacacccgaggtgacctgcgtggtggtggacgtgtcccacgaggatccagaggtgcagtttaactggtacgtggatggcgtggaggtgcataatgctaagaccaagcccagggaggagcagttcaactccacatttcgggtggtgagcgtgctgaccgtggtgcaccaggactggctgaacggcaaggagtataagtgtaaggtgagcaataagggcctgcccgcccctatcgagaagacaatctctaagaccaagggccagcctagagagccacaggtgtacaccctgcccccttctcgcgaggagatgacaaagaaccaggtgtccctgacctgcctggtgaagggcttctatcctagcgacatcgctgtggagtgggagtctaatggccagccagagaacaattacaagaccacaccacccatgctggacagcgatggctctttctttctgtattctaagctgacagtggataagtccaggtggcagcagggcaacgtgtttagctgctctgtgatgcatgaggccctgcacaatcattacacccagaagtccctgagcctgtctccaggcaag

SEQ ID NO: 62 - DNA, 642 bp, Artificial Sequence
  Synthetic polynucleotide
gatatccagatgacacagtccccttccagcctgtctgcctccgtgggcgacagagtgaccatcacatgtcgcgcctcccaggagatctctggctacctgtcctggctgcagcagaagccaggcaaggctcccaagcgcctgatctatgctgcctccaccctggactctggagtgccttccaggttcagcggctctcggtccggcacagagtacaccctgacaatctcttccctgcagcctgaggatttcgccacctactattgcctgcagtacgcttcctatccactgacctttggcggcggcacaaaggtggagatcaagaggacagtggccgctccatccgtgttcatctttccccctagcgacgagcagctgaagagcggcaccgcctctgtggtgtgcctgctgaacaatttctaccccagggaggccaaggtgcagtggaaggtggataacgctctgcagagcggcaattctcaggagtccgtgaccgagcaggacagcaaggattctacatattccctgagctctaccctgacactgagcaaggccgattacgagaagcacaaggtgtatgcttgcgaggtgacccatcagggcctgtccagcccagtgacaaagtcttttaacaggggcgagtgt

SEQ ID NO: 63 - DNA, 21 bp, Artificial Sequence
  Synthetic polynucleotide
catcagccctaatccatctga

SEQ ID NO: 64 - DNA, 21 bp, Artificial Sequence
  Synthetic polynucleotide
cgcgactaacaatcaaagtga

SEQ ID NO: 65 - DNA, 24 bp, Artificial Sequence
  Synthetic polynucleotide
ctaggccacagaattgaaagatct

SEQ ID NO: 66 - DNA, 25 bp, Artificial Sequence
  Synthetic polynucleotide
gtaggtggaaattctagcatcatcc